European Patent Specification EP 3 294 899 B1, published October 15, 2025. Title: PROCEDE DE PRODUCTION DE PROTEINES D'INTERET A PARTIR D'UNE STRUCTURE VEGETALE. Applicant: UNIVERSITE DE PICARDIE JULES VERNES. The sequence listing filed with the application follows.

SEQUENCE LISTING (2 sequences)

SEQ ID NO: 1 - DNA, 13583 bp, artificial sequence
  pRD400-gfp
ccgggctggttgccctcgccgctgggctggcggccgtctatggccctgcaaacgcgccagaaacgccgtcgaagccgtgtgcgagacaccgcggccgccggcgttgtggatacctcgcggaaaacttggccctcactgacagatgaggggcggacgttgacacttgaggggccgactcacccggcgcggcgttgacagatgaggggcaggctcgatttcggccggcgacgtggagctggccagcctcgcaaatcggcgaaaacgcctgattttacgcgagtttcccacagatgatgtggacaagcctggggataagtgccctgcggtattgacacttgaggggcgcgactactgacagatgaggggcgcgatccttgacacttgaggggcagagtgctgacagatgaggggcgcacctattgacatttgaggggctgtccacaggcagaaaatccagcatttgcaagggtttccgcccgtttttcggccaccgctaacctgtcttttaacctgcttttaaaccaatatttataaaccttgtttttaaccagggctgcgccctgtgcgcgtgaccgcgcacgccgaaggggggtgcccccccttctcgaaccctcccggcccgctaacgcgggcctcccatccccccaggggctgcgcccctcggccgcgaacggcctcaccccaaaaatggcagcgctggcagtccttgccattgccgggatcggggcagtaacgggatgggcgatcagcccgagcgcgacgcccggaagcattgacgtgccgcaggtgctggcatcgacattcagcgaccaggtgccgggcagtgagggcggcggcctgggtggcggcctgcccttcacttcggccgtcggggcattcacggacttcatggcggggccggcaatttttaccttgggcattcttggcatagtggtcgcgggtgccgtgctcgtgttcgggggtgcgataaacccagcgaaccatttgaggtgataggtaagattataccgaggtatgaaaacgagaattggacctttacagaattactctatgaagcgccatatttaaaaagctaccaagacgaagaggatgaagaggatgaggaggcagattgccttgaatatattgacaatactgataagataatatatcttttatatagaagatatcgccgtatgtaaggatttcagggggcaaggcataggcagcgcgcttatcaatatatctatagaatgggcaaagcataaaaacttgcatggactaatgcttgaaacccaggacaataaccttatagcttgtaaattctatcataattgggtaatgactccaacttattgatagtgttttatgttcagataatgcccgatgactttgtcatgcagctccaccgattttgagaacgacagcgacttccgtcccagccgtgccaggtgctgcctcagattcaggttatgccgctcaattcgctgcgtatatcgcttgctgattacgtgcagctttcccttcaggcgggattcatacagcggccagccatccgtcatccatatcaccacgtcaaagggtgacagcaggctcataagacgccccagcgtcgccatagtgcgttcaccgaatacgtgcgcaacaaccgtcttccggagactgtcatacgcgtaaaacagccagcgctggcgcgatttagccccgacatagccccactgttcgtccatttccgcgcagacgatgacgtcactgcccggctgtatgcgcgaggttaccgactgcggcctgagttttttaagtgacgtaaaatcgtgttgaggccaacgcccataatgcgggctgttgcccggcatccaacgccattcatggccatatcaatgattttctggtgcgtaccgggttgagaagcggtgtaagtgaactgcagttgccatgttttacggcagtgagagcagagatagcgctgatgtccggcggtgcttttgccgttacgcaccaccccgtcagtagctgaacaggagggacagctgatagacacagaagccactggagcacctcaaaaacaccatcatacactaaatcagtaagttggcagcatcacccataattgtggtttcaaaatcggctccgtcgatactatgttatacgccaactttgaaaacaactttgaaaaagctgttttctggtatttaaggttttagaatgcaaggaacagtgaattggagttcgtcttgttataattagcttcttggggtatctttaaatactgtagaaaagaggaaggaaataataaatggctaaaatgagaatatcaccggaattgaaaaaactgatcgaaaaataccgctgcgtaaaagatacggaaggaatgtctcctgctaaggtatataagctggtgggagaaaatgaaaacctatatttaaaaatgacggacagccggtataaagggaccacctatgatgtggaacgggaaaaggacatgatgctatggctggaaggaaagctgcctgttccaaaggtcctgcactttgaacggcatgatggctggagcaatctgctcatgagtgaggccgatggcgtcctttgctcggaagagtatgaagatgaacaaagccctgaaaagattatcgagctgtatgcggagtgcatcaggctctttcactccatcgacatatcggattgtccctatacgaatagcttagacagccgcttagccgaattggattacttactgaataacgatctggccgatgtggattgcgaaaactgggaagaagacactccatttaaagatccgcgcgagctgtatgattttttaaagacggaaaagcccgaagaggaacttgtcttttcccacggcgacctgggagacagcaacatctttgtgaaagatggcaaagtaagtggctttattgatcttgggagaagcggcagggcggacaagtggtatgacattgccttctgcgtccggtcgatcagggaggatatcggggaagaacagtatgtcgagctattttttgacttactggggatcaagcctgattgggagaaaataaaatattatattttactggatgaattgttttagtacctagatgtggcgcaacgatgccggcgacaagcaggagcgcaccgacttcttccgcatcaagtgttttggctctcaggccgaggcccacggcaagtatttgggcaaggggtcgctggtattcgtgcagggcaagattcggaataccaagtacgagaaggacggccagacggtctacgggaccgacttcattgccgataaggtggattatctggacaccaaggcaccaggcgggtcaaatcaggaataagggcacattgccccggcgtgagtcggggcaatcccgcaaggagggtgaatgaatcggacgtttgaccggaaggcatacaggcaagaactgatcgacgcggggttttccgccgaggatgccgaaaccatcgcaagccgcaccgtcatgcgtgcgccccgcgaaaccttccagtccgtcggctcgatggtccagcaagctacggccaagatcgagcgcgacagcgtgcaactggctccccctgccctgcccgcgccatcggccgccgtggagcgttcgcgtcgtctcgaacaggaggcggcaggtttggcgaagtcgatgaccatcgacacgcgaggaactatgacgaccaagaagcgaaaaaccgccggcgaggacctggcaaaacaggtcagcgaggccaagcaggccgcgttgctgaaacacacgaagcagcagatcaaggaaatgcagctttccttgttcgatattgcgccgtggccggacacgatgcgagcgatgccaaacgacacggcccgctctgccctgttcaccacgcgcaacaagaaaatcccgcgcgaggcgctgcaaaacaaggtcattttccacgtcaacaaggacgtgaagatcacctacaccggcgtcgagctgcgggccgacgatgacgaactggtgtggcagcaggtgttggagtacgcgaagcgcacccctatcggcgagccgatcaccttcacgttctacgagctttgccaggacctgggctggtcgatcaatggccggtattacacgaaggccgaggaatgcctgtcgcgcctacaggcgacggcgatgggcttcacgtccgaccgcgttgggcacctggaatcggtgtcgctgctgcaccgcttccgcgtcctggaccgtggcaagaaaacgtcccgttgccaggtcctgatcgacgaggaaatcgtcgtgctgtttgctggcgaccactacacgaaattcatatgggagaagtaccgcaagctgtcgccgacggcccgacggatgttcgactatttcagctcgcaccgggagccgtacccgctcaagctggaaaccttccgcctcatgtgcggatcggattccacccgcgtgaagaagtggcgcgagcaggtcggcgaagcctgcgaagagttgcgaggcagcggcctggtggaacacgcctgggtcaatgatgacctggtgcattgcaaacgctagggccttgtggggtcagttccggctgggggttcagcagccagcgctttactggcatttcaggaacaagcgggcactgctcgacgcacttgcttcgctcagtatcgctcgggacgcacggcgcgctctacgaactgccgataaacagaggattaaaattgacaattgtgattaaggctcagattcgacggcttggagcggccgacgtgcaggatttccgcgagatccgattgtcggccctgaagaaagctccagagatgttcgggtccgtttacgagcacgaggagaaaaagcccatggaggcgttcgctgaacggttgcgagatgccgtggcattcggcgcctacatcgacggcgagatcattgggctgtcggtcttcaaacaggaggacggccccaaggacgctcacaaggcgcatctgtccggcgttttcgtggagcccgaacagcgaggccgaggggtcgccggtatgctgctgcgggcgttgccggcgggtttattgctcgtgatgatcgtccgacagattccaacgggaatctggtggatgcgcatcttcatcctcggcgcacttaatatttcgctattctggagcttgttgtttatttcggtctaccgcctgccgggcggggtcgcggcgacggtaggcgctgtgcagccgctgatggtcgtgttcatctctgccgctctgctaggtagcccgatacgattgatggcggtcctgggggctatttgcggaactgcgggcgtggcgctgttggtgttgacaccaaacgcagcgctagatcctgtcggcgtcgcagcgggcctggcgggggcggtttccatggcgttcggaaccgtgctgacccgcaagtggcaacctcccgtgcctctgctcacctttaccgcctggcaactggcggccggaggacttctgctcgttccagtagctttagtgtttgatccgccaatcccgatgcctacaggaaccaatgttctcggcctggcgtggctcggcctgatcggagcgggtttaacctacttcctttggttccgggggatctcgcgactcgaacctacagttgtttccttactgggctttctcagccccagatctggggtcgatcagccggggatgcatcaggccgacagtcggaacttcgggtccccgacctgtaccattcggtgagcaatggataggggagttgatatcgtcaacgttcacttctaaagaaatagcgccactcagcttcctcagcggctttatccagcgatttcctattatgtcggcatagttctcaagatcgacagcctgtcacggttaagcgagaaatgaataagaaggctgataattcggatctctgcgagggagatgatatttgatcacaggcagcaacgctctgtcatcgttacaatcaacatgctaccctccgcgagatcatccgtgtttcaaacccggcagcttagttgccgttcttccgaatagcatcggtaacatgagcaaagtctgccgccttacaacggctctcccgctgacgccgtcccggactgatgggctgcctgtatcgagtggtgattttgtgccgagctgccggtcggggagctgttggctggctggtggcaggatatattgtggtgtaaacaaattgacgcttagacaacttaataacacattgcggacgtttttaatgtactggggtggtttttcttttcaccagtgagacgggcaacagctgattgcccttcaccgcctggccctgagagagttgcagcaagcggtccacgctggtttgccccagcaggcgaaaatcctgtttgatggtggttccgaaatcggcaaaatcccttataaatcaaaagaatagcccgagatagggttgagtgttgttccagtttggaacaagagtccactattaaagaacgtggactccaacgtcaaagggcgaaaaaccgtctatcagggcgatggcccactacgtgaaccatcacccaaatcaagttttttggggtcgaggtgccgtaaagcactaaatcggaaccctaaagggagcccccgatttagagcttgacggggaaagccggcgaacgtggcgagaaaggaagggaagaaagcgaaaggagcgggcgccattcaggctgcgcaactgttgggaagggcgatcggtgcgggcctcttcgctattacgccagctggcgaaagggggatgtgctgcaaggcgattaagttgggtaacgccagggttttcccagtcacgacgttgtaaaacgacggccagtgaattcgagctcggtacccctactccaaaaatgtcaaagatacagtctcagaagaccaaagggctattgagacttttcaacaaagggtaatttcgggaaacctcctcggattccattgcccagctatctgtcacttcatcgaaaggacagtagaaaaggaaggtggctcctacaaatgccatcattgcgataaaggaaaggctatcattcaagatgcctctgccgacagtggtcccaaagatggacccccacccacgaggagcatcgtggaaaaagaagacgttccaaccacgtcttcaaagcaagtggattgatgtgacatctccactgacgtaagggatgacgcacaatcccacccctactccaaaaatgtcaaagatacagtctcagaagaccaaagggctattgagacttttcaacaaagggtaatttcgggaaacctcctcggattccattgcccagctatctgtcacttcatcgaaaggacagtagaaaaggaaggtggctcctacaaatgccatcattgcgataaaggaaaggctatcattcaagatgcctctgccgacagtggtcccaaagatggacccccacccacgaggagcatcgtggaaaaagaagacgttccaaccacgtcttcaaagcaagtggattgatgtgacatctccactgacgtaagggatgacgcacaatcccactatccttcgcaagacccttcctctatataaggaagttcatttcatttggagaggacagcccaagcttaaaacaacaatgggatacacaaatgtgtccattttattaggcctgttgatggtctttgttacaccgatggtgttcgcagatcccatgcatcatcatcatcaccaccccatggtgagcaagggcgaggagctgttcaccggggtggtgcccatcctggtcgagctggacggcgacgtaaacggccacaagttcagcgtgtccggcgagggcgagggcgatgccacctacggcaagctgaccctgaagttcatctgcaccaccggcaagctgcccgtgccctggcccaccctcgtgaccaccctgacctacggcgtgcagtgcttcagccgctaccccgaccacatgaagcagcacgacttcttcaagtccgccatgcccgaaggctacgtccaggagcgcaccatcttcttcaaggacgacggcaactacaagacccgcgccgaggtgaagttcgagggcgacaccctggtgaaccgcatcgagctgaagggcatcgacttcaaggaggacggcaacatcctggggcacaagctggagtacaactacaacagccacaacgtctatatcatggccgacaagcagaagaacggcatcaaggtgaacttcaagatccgccacaacatcgaggacggcagcgtgcagctcgccgaccactaccagcagaacacccccatcggcgacggccccgtgctgctgcccgacaaccactacctgagcacccagtccgccctgagcaaagaccccaacgagaagcgcgatcacatggtcctgctggagttcgtgaccgccgccgggatcactctcggcatggacgagctgtacaagtaaagcggccgcgactctagaattcgctgaaatcaccagtctctctctacaaatctatctctctctattttctccataaataatgtgtgagtagtttcccgataagggaaattagggttcttatagggtttcgctcatgtgttgagcatataagaaacccttagtatgtatttgtatttgtaaaatacttctatcaataaaatttctaattcctaaaaccaaaatccagtactaaaatccagatcctctagagtcgacctgcaggcatgcaagcttggcgtaatcatggtcatagctgtttcctgtgtgaaattgttatccgctcacaattccacacaacatacgagccggaagcataaagtgtaaagcctggggtgcctaatgagtgagctaactcacattaattgcgttgcgctcactgcccgctttccagtcgggaaacctgtcgtgccagctgcattaatgaatcggccaacgcgcggggagaggcggtttgcgtattgggccaaagacaaaagggcgacattcaaccgattgagggagggaaggtaaatattgacggaaattattcattaaaggtgaattatcaccgtcaccgacttgagccatttgggaattagagccagcaaaatcaccagtagcaccattaccattagcaaggccggaaacgtcaccaatgaaaccatcgatagcagcaccgtaatcagtagcgacagaatcaagtttgcctttagcgtcagactgtagcgcgttttcatcggcattttcggtcatagcccccttattagcgtttgccatcttttcataatcaaaatcaccggaaccagagccaccaccggaaccgcctccctcagagccgccaccctcagaaccgccaccctcagagccaccaccctcagagccgccaccagaaccaccaccagagccgccgccagcattgacaggaggcccgatctagtaacatagatgacaccgcgcgcgataatttatcctagtttgcgcgctatattttgttttctatcgcgtattaaatgtataattgcgggactctaatcataaaaacccatctcataaataacgtcatgcattacatgttaattattacatgcttaacgtaattcaacagaaattatatgataatcatcgcaagaccggcaacaggattcaatcttaagaaactttattgccaaatgtttgaacgatcggggatcatccgggtctgtggcgggaactccacgaaaatatccgaacgcagcaagatatcgcggtgcatctcggtcttgcctgggcagtcgccgccgacgccgttgatgtggacgccgggcccgatcatattgtcgctcaggatcgtggcgttgtgcttgtcggccgttgctgtcgtaatgatatcggcaccttcgaccgcctgttccgcagagatcccgtgggcgaagaactccagcatgagatccccgcgctggaggatcatccagccggcgtcccggaaaacgattccgaagcccaacctttcatagaaggcggcggtggaatcgaaatctcgtgatggcaggttgggcgtcgcttggtcggtcatttcgaaccccagagtcccgctcagaagaactcgtcaagaaggcgatagaaggcgatgcgctgcgaatcgggagcggcgataccgtaaagcacgaggaagcggtcagcccattcgccgccaagctcttcagcaatatcacgggtagccaacgctatgtcctgatagcggtccgccacacccagccggccacagtcgatgaatccagaaaagcggccattttccaccatgatattcggcaagcaggcatcgccatgggtcacgacgagatcctcgccgtcgggcatgcgcgccttgagcctggcgaacagttcggctggcgcgagcccctgatgctcttcgtccagatcatcctgatcgacaagaccggcttccatccgagtacgtgctcgctcgatgcgatgtttcgcttggtggtcgaatgggcaggtagccggatcaagcgtatgcagccgccgcattgcatcagccatgatggatactttctcggcaggagcaaggtgagatgacaggagatcctgccccggcacttcgcccaatagcagccagtcccttcccgcttcagtgacaacgtcgagcacagctgcgcaaggaacgcccgtcgtggccagccacgatagccgcgctgcctcgtcctgcagttcattcagggcaccggacaggtcggtcttgacaaaaagaaccgggcgcccctgcgctgacagccggaacacggcggcatcagagcagccgattgtctgttgtgcccagtcatagccgaatagcctctccacccaagcggccggagaacctgcgtgcaatccatcttgttcaatcatgcgaaacgatccagatccggtgcagattatttggattgagagtgaatatgagactctaattggataccgaggggaatttatggaacgtcagtggagcatttttgacaagaaatatttgctagctgatagtgaccttaggcgacttttgaacgcgcaataatggtttctgacgtatgtgcttagctcattaaactccagaaacccgcggctgagtggctccttcaacgttgcggttctgtcagttccaaacgtaaaacggcttgtcccgcgtcatcggcgggggtcataacgtgactcccttaattctccgctcatgatcagattgtcgtttcccgccttcagtttaaactatcagtgtttgacaggatatattggcgggtaaacctaagagaaaagagcgtttattagaataatcggatatttaaaagggcgtgaaaaggtttatccgttcgtccatttgtatgtgcatgccaaccacagggttccccagatctggcgccggccagcgagacgagcaagattggccgccgcccgaaacgatccgacagcgcgcccagcacaggtgcgcaggcaaattgcaccaacgcatacagcgccagcagaatgccatagtgggcggtgacgtcgttcgagtgaaccagatcgcgcaggaggcccggcagcaccggcataatcaggccgatgccgacagcgtcgagcgcgacagtgctcagaattacgatcaggggtatgttgggtttcacgtctggcctccggaccagcctccgctggtccgattgaacgcgcggattctttatcactgataagttggtggacatattatgtttatcagtgataaagtgtcaagcatgacaaagttgcagccgaatacagtgatccgtgccgccctggacctgttgaacgaggtcggcgtagacggtctgacgacacgcaaactggcggaacggttgggggttcagcagccggcgctttactggcacttcaggaacaagcgggcgctgctcgacgcactggccgaagccatgctggcggagaatcatacgcattcggtgccgagagccgacgacgactggcgctcatttctgatcgggaatgcccgcagcttcaggcaggcgctgctcgcctaccgcgatggcgcgcgcatccatgccggcacgcgaccgggcgcaccgcagatggaaacggccgacgcgcagcttcgcttcctctgcgaggcgggtttttcggccggggacgccgtcaatgcgctgatgacaatcagctacttcactgttggggccgtgcttgaggagcaggccggcgacagcgatgccggcgagcgcggcggcaccgttgaacaggctccgctctcgccgctgttgcgggccgcgatagacgccttcgacgaagccggtccggacgcagcgttcgagcagggactcgcggtgattgtcgatggattggcgaaaaggaggctcgttgtcaggaacgttgaaggaccgagaaagggtgacgattgatcaggaccgctgccggagcgcaacccactcactacagcagagccatgtagacaacatcccctccccctttccaccgcgtcagacgcccgtagcagcccgctacgggctttttcatgccctgccctagcgtccaagcctcacggccgcgctcggcctctctggcggccttctggcgctcttccgcttcctcgctcactgactcgctgcgctcggtcgttcggctgcggcgagcggtatcagctcactcaaaggcggtaatacggttatccacagaatcaggggataacgcaggaaagaacatgtgagcaaaaggccagcaaaaggccaggaaccgtaaaaaggccgcgttgctggcgtttttccataggctccgcccccctgacgagcatcacaaaaatcgacgctcaagtcagaggtggcgaaacccgacaggactataaagataccaggcgtttccccctggaagctccctcgtgcgctctcctgttccgaccctgccgcttaccggatacctgtccgcctttctcccttcgggaagcgtggcgcttttccgctgcataaccctgcttcggggtcattatagcgattttttcggtatatccatcctttttcgcacgatatacaggattttgccaaagggttcgtgtagactttccttggtgtatccaacggcgtcagccgggcaggataggtgaagtaggcccacccgcgagcgggtgttccttcttcactgtcccttattcgcacctggcggtgctcaacgggaatcctgctctgcgaggctggccggctaccgccggcgtaacagatgagggcaagcggatggctgatgaaaccaagccaaccaggaagggcagcccacctatcaaggtgtactgccttccagacgaacgaagagcgattgaggaaaaggcggcggcggccggcatgagcctgtcggcctacctgctggccgtcggccagggctacaaaatcacgggcgtcgtggactatgagcacgtccgcgagctggcccgcatcaatggcgacctgggccgcctgggcggcctgctgaaactctggctcaccgacgacccgcgcacggcgcggttcggtgatgccacgatcctcgccctgctggcgaagatcgaagagaagcaggacgagcttggcaaggtcatgatgggcgtggtccgcccgagggcagagccatgacttttttagccgctaaaacggccggggggtgcgcgtgattgccaagcacgtccccatgcgctccatcaagaagagcgacttcgcggagctggtgaagtacatcaccgacgagcaaggcaagaccgagcgcctttgcgacgctca

SEQ ID NO: 2 - DNA, 1215 bp, artificial sequence
  GL-SP
ccatgggttatacaaacgtttcaatcctattaggcttgttgatggttttcgtcactcctatggtatttgcactcttcgggaagttacacccaggctccccagaggtaactatgaacatatcacagatgattacatattggggatatccaaatgaggaatatgaagtggtcacggaggacggatacattttggaagtgaacagaataccgtacgggaagaagaacagtggaaacaccggtcaacgtcccgtcgtgttccttcaacatggacttctagcaagtgctactaattggattagcaacttgccgaataactcacttgcctttatcttagcagatgcaggctatgatgtttggctgggaaacagtagaggcaatacatgggcaaggcgtaatctttactactctccggatagtgttgagttttgggcttttagcttcgacgaaatggcgaagtacgatcttccggctactattgactttatcgttaagaaaacgggacagaagcagttacattatgtgggtcattcccaggggaccactatcggattcatcgccttttctacgaacccttccctcgcaaaacgaatcaaaaccttttacgctctcgcgcctgttgcaactgtgaaatacacgaagtctctgattaacaaactgagatttgttcctcaatctttgttcaagtttatctttggtgataagattttctatcctcacaacttctttgatcaatttcttgccacagaagtttgctcgcgagaaatgctcaatctcctatgttccaacgctttgtttatcatatgtggattcgattcgaagaatttcaatacttctagattggatgtgtatttgtcacacaatccagctgggacctctgttcagaatatgttccattggacacaagctgtgaaaagcggaaagtttcaagcttatgattggggttctcccgtccagaataggatgcactatgaccagtcacaacctccttactacaacgtaacagcgatgaacgtgccaattgctgtttggaatggtggtaaagacctactagctgatccacaagatgtcggtctgcttcttcctaaacttcccaatttgatataccataaagaaattccattctataaccatcttgacttcatatgggctatggatgcaccgcaagaggtctacaatgatatagtatcgatgattagcgaggataagaaatgaattc